European Patent Application EP 4 527 918 A1, published March 26, 2025. Title: MICROORGANISM BELONGING TO GENUS AKKERMANSIA. Applicant: Otsuka Pharmaceutical Co., Ltd. The sequence listing filed with the application follows.

SEQUENCE LISTING (3 sequences)

SEQ ID NO: 1 - DNA, 1433 bp, Akkermansia_muciniphila
  source 1..1433: mol_type = genomic DNA
aacgaacgctggcggcgtggataagacatgcaagtcgaacgagagaattgctagcttgctaataattctctagtggcgcacgggtgagtaacacgtgagtaacctgcccccgagagcgggatagccctgggaaactgggattaataccgcatagtatcgaaagattaaagcagcaatgcgcttggggatgggctcgcggcctattagttagttggtgaggtaacggctcaccaaggcgatgacgggtagccggtctgagaggatgtccggccacactggaactgagacacggtccagacacctacgggtggcagcagtcgagaatcattcacaatgggggaaaccctgatggtgcgacgccgcgtgggggaatgaaggtcttcggattgtaaacccctgtcatgtgggagcaaattaaaaagatagtaccacaagaggaagagacggctaactctgtgccagcagccgcggtaatacagaggtctcaagcgttgttcggaatcactgggcgtaaagcgtgcgtaggctgtttcgtaagtcgtgtgtgaaaggcgcgggctcaacccgcggacggcacatgatactgcgagactagagtaatggagggggaaccggaattctcggtgtagcagtgaaatgcgtagatatcgagaggaacactcgtggcgaaggcgggttcctggacattaactgacgctgaggcacgaaggccaggggagcgaaagggattagatacccctgtagtcctggcagtaaacggtgcacgcttggtgtgcggggaatcgaccccctgcgtgccggagtaacgcgttaagcgtgccgcctggggagtacggtcgcaagattaaaactcaaagaaattgacggggacccgcacaagcggtggagtatgtggcttaattcgatgcaacgcgaagaaccttacctgggcttgacatgtaatgaacaacatgtgaaagcatgcgactcttcggaggcgttacacaggtgctgcatggccgtcgtcagctcgtgtcgtgagatgtttggttaagtccagcaacgagcgcaacccctgttgccagttaccagcacgtgaaggtggggactctggcgagactgcccagatcaactgggaggaaggtggggacgacgtcaggtcagtatggcccttatgcccagggctgcacacgtactacaatgcccagtacagagggggccgaagccgcgaggcggaggaaatcctaaaaactgggcccagttcggactgtaggctgcaacccgcctacacgaagccggaatcgctagtaatggcgcatcagctacggcgccgtgaatacgttcccgggtcttgtacacaccgcccgtcacatcatggaagctggtcgcacccgaagtatctgaagccaaccgcaaggaggcagggtcctaaggtgagactggtaactgggatg

SEQ ID NO: 2 - DNA, 1438 bp, Akkermansia_glycaniphila
  source 1..1438: mol_type = genomic DNA
aacgaacgctggcggcgtggataagacatgcaagtcgaacggagaagcaatagcttgctaatgcttcttagtggcgcacgggtgagtaacacgtgagcaacctgccttcgagacgggaatagccctgggaaaccgggattaatgcccgatagactcgcaagagtaaacgcagcaatgcgcttgaagaggggctcgcggcctattagttagttggtgaggtaacggctcaccaaggcgatgacgggtagccggtctgagaggatgtccggccacactggaactgagacacggtccagacacctacgggtggcagcagtcgagaatcattcacaatgggggaaaccctgatggtgcgacgccgcgtgggggaagaaggtcttcggattgtaaacccctgtcatgtgggagcaaggcgcaagcttgatagtaccacaagaggaagagacggctaactctgtgccagcagccgcggtaatacagaggtctcaagcgttgttcggaatcactgggcgtaaagggtacgtaggctgcatcataagtcgggcgtgaaaggcaggggctcaacccctggagtgcgcttgatactgtgatgctagagtcatggagggggaaccggaactctcggtgtagcagtgaaatgcgtagatatcgagaagaacactcgtggcgaaggcgggttcctggacatgtactgacgctgaggtacgaaggctaggggagcgaaagggattagatacccctgtagtcctagcagtaaacggtgcacgcttggtgtgtggggaatcgaccccccacgtgccggagcaaacgcgttaagcgtgccgcctggggagtacggtcgcaagattaaaactcaaagaaattgacggggacccgcacaagcggtggagtatgtggcttaattcgatgcaacgcgaagaaccttacctgggcttgacatgtgatgaacaacatgtgaaagcatgtgacacctcggtggcgtcacacaggtgctgcatggccgtcgtcagctcgtgtcgtgagatgtttggttaagtccagcaacgagcgcaacccctgttgccagttaccagcacgttatggtggggactctggcgagactgcccagatcaactgggaggaaggtggggacgacgtcaggtcagtatggcccttatgcccagggctgcacacgtactacaatgcccagtacagagggtaccgaacccgcgagggggaggcaatccatgaaaactgggcccagttcggattgtaggctgcaactcgcctacatgaagatggaatcgctagtaatggcgcatcagctacggcgccgtgaatacgttcccgggtcttgtacacaccgcccgtcacatcatggaagccggtcgcacccgaagtatctgaagccaaccgcaaggaggcagggtcctaaggtgagactggtaactgggatgaa

SEQ ID NO: 3 - DNA, 1437 bp, Akkermansia
  source 1..1437: mol_type = genomic DNA
aacgaacgctggcggcgtggataagacatgcaagtcgaacgggagaattgctagcttgctaataattctctagtggcgcacgggtgagtaacacgtgagtaacctgcctcttagtgggggatagccctgggaaaccgggattaataccgcatacgattgaaagatcaaagcagcaatgcgctaggagatgggctcgcggcctattagttagttggtgaggtaacggctcaccaaggcgatgacgggtagccggtctgagaggatgtccggccacactggaactgagacacggtccagacacctacgggtggcagcagtcgagaatcattcacaatgggggcaaccctgatggtgcgacgccgcgtgggggaatgaaggtcttcggattgtaaacccctgtcatgtgggagcaaattaaaaagatagtaccacaagaggaagagacggctaactctgtgccagcagccgcggtaatacagaggtctcaagcgttgttcggaatcactgggcgtaaagcgtgcgtaggctgtttcgtaagtcgtgtgtgaaaggcaggggctcaacccctggattgcacatgatactgcgagactagagtaatggagggggaaccggaattctcggtgtagcagtgaaatgcgtagatatcgagaggaacactcgtggcgaaggcgggttcctggacattaactgacgctgaggcacgaaggccaggggagcgaaagggattagatacccctgtagtcctggcagtaaacggtgcacgcttggtgtgcggggaatcgaccccctgcgtgccggagctaacgcgttaagcgtgccgcctggggagtacggtcgcaagattaaaactcaaagaaattgacggggacccgcacaagcggtggagtatgtggcttaattcgatgcaacgcgaagaaccttacctgggcttgacatgtaatgaacaacatgtgaaagcatgcgactcttcggaggcgttacacaggtgctgcatggccgtcgtcagctcgtgtcgtgagatgtttggttaagtccagcaacgagcgcaacccctgttgccagttaccatcgagtaatgtcggggactctggcgagactgcccagatcaactgggaggaaggtggggacgacgtcaggtcagtatggcccttatgcccagggctgcacacgtactacaatgcccagtacagagggggccgaagccgcgaggcggaggaaatcctgaaaactgggcccagttcggactgtaggctgcaacccgcctacacgaagccggaatcgctagtaatggcgcatcagctacggcgccgtgaatacgttcccgggtcttgtacacaccgcccgtcacatcatggaagccggtcgcacccgaagtatctgaagccaaccgcaaggaggcagggtcctaaggtgagactggtaactgggatgaag